European Patent Application EP 4 234 575 A1, published August 30, 2023. Title: A Cell surface antigen of activated immune cell and the use thereof. Applicant: Good T Cells, Inc. The sequence listing filed with the application follows.

SEQUENCE LISTING (52 sequences)

SEQ ID NO: 1 - protein, 759 aa, Homo sapiens
GPRAPCAAACTCAGDSLDCGGRGLAALPGDLPSWTRSLNLSYNKLSEIDPAGFEDLPNLQEVYLNNNELTAVPSLGAASSHVVSLFLQHNKIRSVEGSQLKAYLSLEVLDLSLNNITEVRNTCFPHGPPIKELNLAGNRIGTLELGAFDGLSRSLLTLRLSKNRITQLPVRAFKLPRLTQLDLNRNRIRLIEGLTFQGLNSLEVLKLQRNNISKLTDGAFWGLSKMHVLHLEYNSLVEVNSGSLYGLTALHQLHLSNNSIARIHRKGWSFCQKLHELVLSFNNLTRLDEESLAELSSLSVLRLSHNSISHIAEGAFKGLRSLRVLDLDHNEISGTIEDTSGAFSGLDSLSKLTLFGNKIKSVAKRAFSGLEGLEHLNLGGNAIRSVQFDAFVKMKNLKELHISSDSFLCDCQLKWLPPWLIGRMLQAFVTATCAHPESLKGQSIFSVPPESFVCDDFLKPQIITQPETTMAMVGKDIRFTCSAASSSSSPMTFAWKKDNEVLTNADMENFVHVHAQDGEVMEYTTILHLRQVTFGHEGRYQCVITNHFGSTYSHKARLTVNVLPSFTKTPHDITIRTTTVARLECAATGHPNPQIAWQKDGGTDFPAARERRMHVMPDDDVFFITDVKIDDAGVYSCTAQNSAGSISANATLTVLETPSLVVPLEDRVVSVGETVALQCKATGNPPPRITWFKGDRPLSLTERHHLTPDNQLLVVQNVVAEDAGRYTCEMSNTLGTERAHSQLSVLPAAGCRKDGTTVG

SEQ ID NO: 2 - DNA, 2397 bp, Homo sapiens
ggcccgcgggcgccctgcgcggccgcctgcacttgcgctggggactcgctggactgcggtgggcgcgggctggctgcgttgcccggggacctgccctcctggacgcggagcctaaacctgagttacaacaaactctctgagattgaccctgctggttttgaggacttgccgaacctacaggaagtgtacctcaataataatgagttgacagcggtaccatccctgggcgctgcttcatcacatgtcgtctctctctttctgcagcacaacaagattcgcagcgtggaggggagccagctgaaggcctacctttccttagaagtgttagatctgagtttgaacaacatcacggaagtgcggaacacctgctttccacacggaccgcctataaaggagctcaacctggcaggcaatcggattggcaccctggagttgggagcatttgatggtctgtcacggtcgctgctaactcttcgcctgagcaaaaacaggatcacccagcttcctgtaagagcattcaagctacccaggctgacacaactggacctcaatcggaacaggattcggctgatagagggcctcaccttccaggggctcaacagcttggaggtgctgaagcttcagcgaaacaacatcagcaaactgacagatggggccttctggggactgtccaagatgcatgtgctgcacctggagtacaacagcctggtagaagtgaacagcggctcgctctacggcctcacggccctgcatcagctccacctcagcaacaattccatcgctcgcattcaccgcaagggctggagcttctgccagaagctgcatgagttggtcctgtccttcaacaacctgacacggctggacgaggagagcctggccgagctgagcagcctgagtgtcctgcgtctcagccacaattccatcagccacattgcggagggtgccttcaagggactcaggagcctgcgagtcttggatctggaccataacgagatttcgggcacaatagaggacacgagcggcgccttctcagggctcgacagcctcagcaagctgactctgtttggaaacaagatcaagtctgtggctaagagagcattctcggggctggaaggcctggagcacctgaaccttggagggaatgcgatcagatctgtccagtttgatgcctttgtgaagatgaagaatcttaaagagctccatatcagcagcgacagcttcctgtgtgactgccagctgaagtggctgcccccgtggctaattggcaggatgctgcaggcctttgtgacagccacctgtgcccacccagaatcactgaagggtcagagcattttctctgtgccaccagagagtttcgtgtgcgatgacttcctgaagccacagatcatcacccagccagaaaccaccatggctatggtgggcaaggacatccggtttacatgctcagcagccagcagcagcagctcccccatgacctttgcctggaagaaagacaatgaagtcctgaccaatgcagacatggagaactttgtccacgtccacgcgcaggacggggaagtgatggagtacaccaccatcctgcacctccgtcaggtcactttcgggcacgagggccgctaccaatgtgtcatcaccaaccactttggctccacctattcacataaggccaggctcaccgtgaatgtgttgccatcattcaccaaaacgccccacgacataaccatccggaccaccaccgtggcccgcctcgaatgtgctgccacaggtcacccaaaccctcagattgcctggcagaaggatggaggcacggatttccccgctgcccgtgagcgacgcatgcatgtcatgccggatgacgacgtgtttttcatcactgatgtgaaaatagatgacgcaggggtttacagctgtactgctcagaactcagccggttctatttcagctaatgccaccctgactgtcctagagaccccatccttggtggtccccttggaagaccgtgtggtatctgtgggagaaacagtggccctccaatgcaaagccacggggaaccctccgccccgcatcacctggttcaagggggaccgcccgctgagcctcactgagcggcaccacctgacccctgacaaccagctcctggtggttcagaacgtggtggcagaggatgcgggccgatatacctgtgagatgtccaacaccctgggcacggagcgagctcacagccagctgagcgtcctgcccgcagcaggctgcaggaaggatgggaccacggtaggcatcttcaccattgctgtcgtgagcagcatcgtcctgacgtcactggtctgggtgtgcatcatctaccagaccaggaagaagagtgaagagtacagtgtcaccaacacagatgaaaccgtc

SEQ ID NO: 3 - protein, 761 aa, Mus musculus
QAGPRAPCAAACTCAGDSLDCSGRGLATLPRDLPSWTRSLNLSYNRLSEIDSAAFEDLTNLQEVYLNSNELTAIPSLGAASIGVVSLFLQHNKILSVDGSQLKSYLSLEVLDLSSNNITEIRSSCFPNGLRIRELNLASNRISILESGAFDGLSRSLLTLRLSKNRITQLPVKAFKLPRLTQLDLNRNRIRLIEGLTFQGLDSLEVLRLQRNNISRLTDGAFWGLSKMHVLHLEYNSLVEVNSGSLYGLTALHQLHLSNNSISRIQRDGWSFCQKLHELILSFNNLTRLDEESLAELSSLSILRLSHNAISHIAEGAFKGLKSLRVLDLDHNEISGTIEDTSGAFTGLDNLSKLTLFGNKIKSVAKRAFSGLESLEHLNLGENAIRSVQFDAFAKMKNLKELYISSESFLCDCQLKWLPPWLMGRMLQAFVTATCAHPESLKGQSIFSVLPDSFVCDDFPKPQIITQPETTMAVVGKDIRFTCSAASSSSSPMTFAWKKDNEVLANADMENFAHVRAQDGEVMEYTTILHLRHVTFGHEGRYQCIITNHFGSTYSHKARLTVNVLPSFTKIPHDIAIRTGTTARLECAATGHPNPQIAWQKDGGTDFPAARERRMHVMPDDDVFFITDVKIDDMGVYSCTAQNSAGSVSANATLTVLETPSLAVPLEDRVVTVGETVAFQCKATGSPTPRITWLKGGRPLSLTERHHFTPGNQLLVVQNVMIDDAGRYTCEMSNPLGTERAHSQLSILPTPGCRKDGTTVG

SEQ ID NO: 4 - DNA, 2283 bp, Mus musculus
caggctggcccgcgggccccctgcgcggccgcctgcacttgcgccggggactcgctggactgcagtgggcgcgggctggcgacgctgccccgggacctgccctcctggacgcgcagcctaaacctgagttataacagactctccgagatcgactctgctgcttttgaggacttgacgaatctgcaggaagtgtacctcaacagcaatgagctgacagccataccatcactgggcgctgcttccataggagttgtctctctctttttgcagcacaacaagatccttagtgtggatgggagccagctgaagtcgtacctgtccttggaagtgctggatctgagttccaacaacatcacggaaattcggagctcctgtttcccgaacggcctgcgtataagggaactcaacttggcgagcaaccgcatcagcatcctggagtctggagcatttgatggtctgtcgcggtcactgctgactctccgtctgagcaaaaacaggatcacccagcttcctgtgaaagcgttcaagctacccaggctgacacaactagacctgaatcggaatcggattcggctgattgaaggcctcacgttccaggggctcgacagcttagaggtgctgaggcttcagaggaacaacatcagcaggctgacggacggggccttctgggggctgtctaagatgcacgtgctgcacctggagtacaacagtctggtggaagtgaacagtggctccctctatggcctcacagccctgcaccagctgcacctcagcaacaactccatctctcgaattcagcgtgatggctggagcttctgccaaaagctgcatgagttgattctgtccttcaacaacctcacgcggctggatgaggagagtctagcggagttgagcagcctcagtatcctgcgcctcagtcacaacgccatcagtcacattgctgaaggcgccttcaagggactcaagagtctgcgggtcttggacctggaccataacgagatctcgggtacaatcgaggataccagtggtgcctttacggggcttgacaacctcagcaagctgactctgtttggaaacaagatcaaatctgtggctaagagagccttctcgggcctggaaagcctggaacacctgaaccttggagagaatgcaatcaggtctgtccagtttgatgcctttgcaaagatgaagaaccttaaagagctctacatcagcagtgagagcttcctgtgtgactgccagctcaagtggctgcccccatggctaatgggtaggatgctgcaggcctttgtgacagccacctgtgcccatccagagtcgctgaagggccagagcattttctcagtgctgccagacagctttgtgtgtgatgactttccaaagccacagatcatcacccagcctgagacgaccatggctgtggtgggcaaggacatccgtttcacatgctccgcagccagcagcagcagctcaccaatgaccttcgcctggaagaaggacaatgaggtcctggccaatgcagacatggagaactttgcccacgtccgtgcacaggacggcgaagtgatggagtataccactatcctgcacctccgtcacgtcacctttgggcacgagggccgctaccagtgtatcatcacaaaccactttggctccacatactcccacaaagccaggctcactgtgaatgtgttgccatcattcactaaaataccccatgacattgccatccggactggcaccacagcccgcctcgagtgtgctgccacgggccaccctaaccctcagattgcctggcagaaggatggaggcaccgatttcccggcagctcgtgagcgacgcatgcatgttatgccagacgatgatgtgttcttcatcactgatgtgaaaatagacgacatgggggtctacagctgcactgcccagaactcggcaggctcggtttcagccaacgctaccctcacagtcttagaaactccatccttggcagtgcctctggaagaccgtgtggtaactgtgggagaaacagtggccttccagtgcaaagcaaccgggagccccacaccacgcatcacctggcttaagggaggtcgcccattgagcctcacagagcgccaccatttcactccaggcaaccagctgctggttgttcagaatgtgatgatagacgatgcagggcggtatacctgtgagatgtctaatcccctgggcactgagcgagcacatagccagctgagcattttacctacccctggctgccggaaggatgggaccaccgtaggc

SEQ ID NO: 5 - protein, 8 aa, Artificial Sequence
  GTC110-01 heavy chain CDR1
GFTFSDYD

SEQ ID NO: 6 - protein, 9 aa, Artificial Sequence
  GTC110-01 heavy chain CDR2
WISHGGGSI

SEQ ID NO: 7 - protein, 20 aa, Artificial Sequence
  GTC110-01 heavy chain CDR3
ARGLGLCKTGLCYYYDAMDV

SEQ ID NO: 8 - protein, 8 aa, Artificial Sequence
  GTC110-01 light chain CDR1
SSNIGNNS

SEQ ID NO: 9 - protein, 3 aa, Artificial Sequence
  GTC110-01 light chain CDR2
ADN

SEQ ID NO: 10 - protein, 11 aa, Artificial Sequence
  GTC110-01 light chain CDR3
AAWDSSLSAYV

SEQ ID NO: 11 - protein, 8 aa, Artificial Sequence
  GTC110-02 heavy chain CDR1
GFTFSDYY

SEQ ID NO: 12 - protein, 9 aa, Artificial Sequence
  GTC110-02 heavy chain CDR2
GISHDSGSK

SEQ ID NO: 13 - protein, 9 aa, Artificial Sequence
  GTC110-02 heavy chain CDR3
ARHWTTFDY

SEQ ID NO: 14 - protein, 8 aa, Artificial Sequence
  GTC110-02 light chain CDR1
SSNIGSNN

SEQ ID NO: 15 - protein, 3 aa, Artificial Sequence
  GTC110-02 light chain CDR2
ANS

SEQ ID NO: 16 - protein, 11 aa, Artificial Sequence
  GTC110-02 light chain CDR3
GAWDYSLSAYV

SEQ ID NO: 17 - protein, 8 aa, Artificial Sequence
  GTC110-03 heavy chain CDR1
GFTFSNYA

SEQ ID NO: 18 - protein, 9 aa, Artificial Sequence
  GTC110-03 heavy chain CDR2
AIYPGGGSI

SEQ ID NO: 19 - protein, 20 aa, Artificial Sequence
  GTC110-03 heavy chain CDR3
ARDILPCPWGRCYYDYAMDV

SEQ ID NO: 20 - protein, 8 aa, Artificial Sequence
  GTC110-03 light chain CDR1
SSNIGSNT

SEQ ID NO: 21 - protein, 3 aa, Artificial Sequence
  GTC110-03 light chain CDR2
ADN

SEQ ID NO: 22 - protein, 11 aa, Artificial Sequence
  GTC110-03 light chain CDR3
GTWDYSLSGYV

SEQ ID NO: 23 - protein, 8 aa, Artificial Sequence
  GTC110-04 heavy chain CDR1
GFTFSNYA

SEQ ID NO: 24 - protein, 9 aa, Artificial Sequence
  GTC110-04 heavy chain CDR2
VISHGGGST

SEQ ID NO: 25 - protein, 20 aa, Artificial Sequence
  GTC110-04 heavy chain CDR3
ARVISNCHLGVCYYSNGMDV

SEQ ID NO: 26 - protein, 8 aa, Artificial Sequence
  GTC110-04 light chain CDR1
SSNIGNND

SEQ ID NO: 27 - protein, 3 aa, Artificial Sequence
  GTC110-04 light chain CDR2
SDS

SEQ ID NO: 28 - protein, 11 aa, Artificial Sequence
  GTC110-04 light chain CDR3
GTWDYSLSGYV

SEQ ID NO: 29 - protein, 8 aa, Artificial Sequence
  GTC210-01 heavy chain CDR1
GFTFSGYD

SEQ ID NO: 30 - protein, 9 aa, Artificial Sequence
  GTC210-01 heavy chain CDR2
LIYPDSGNK

SEQ ID NO: 31 - protein, 14 aa, Artificial Sequence
  GTC210-01 heavy chain CDR3
ARDAGLSWAGAFDY

SEQ ID NO: 32 - protein, 8 aa, Artificial Sequence
  GTC210-01 light chain CDR1
SSNIGSNY

SEQ ID NO: 33 - protein, 3 aa, Artificial Sequence
  GTC210-01 light chain CDR2
SDS

SEQ ID NO: 34 - protein, 11 aa, Artificial Sequence
  GTC210-01 light chain CDR3
GSWDYSLSAYV

SEQ ID NO: 35 - protein, 8 aa, Artificial Sequence
  GTC210-02 heavy chain CDR1
GFTFSNYY

SEQ ID NO: 36 - protein, 9 aa, Artificial Sequence
  GTC210-02 heavy chain CDR2
GISPGDSST

SEQ ID NO: 37 - protein, 14 aa, Artificial Sequence
  GTC210-02 heavy chain CDR3
AKGLYSNPNEPFDY

SEQ ID NO: 38 - protein, 8 aa, Artificial Sequence
  GTC210-02 light chain CDR1
SSNIGSNY

SEQ ID NO: 39 - protein, 3 aa, Artificial Sequence
  GTC210-02 light chain CDR2
DDS

SEQ ID NO: 40 - protein, 11 aa, Artificial Sequence
  GTC210-02 light chain CDR3
GTWDYSLNGYV

SEQ ID NO: 41 - protein, 8 aa, Artificial Sequence
  GTC210-03 heavy chain CDR1
GFTFSSYD

SEQ ID NO: 42 - protein, 9 aa, Artificial Sequence
  GTC210-03 heavy chain CDR2
GISPDGSNI

SEQ ID NO: 43 - protein, 20 aa, Artificial Sequence
  GTC210-03 heavy chain CDR3
AKVGLRCRYEACSYAYGMDV

SEQ ID NO: 44 - protein, 8 aa, Artificial Sequence
  GTC210-03 light chain CDR1
SSNIGSNY

SEQ ID NO: 45 - protein, 3 aa, Artificial Sequence
  GTC210-03 light chain CDR2
SDS

SEQ ID NO: 46 - protein, 11 aa, Artificial Sequence
  GTC210-03 light chain CDR3
ATWDSSLNGYV

SEQ ID NO: 47 - protein, 8 aa, Artificial Sequence
  GTC210-04 heavy chain CDR1
GFTFSNYD

SEQ ID NO: 48 - protein, 9 aa, Artificial Sequence
  GTC210-04 heavy chain CDR2
SISPSSGSI

SEQ ID NO: 49 - protein, 14 aa, Artificial Sequence
  GTC210-04 heavy chain CDR3
AKDLDAFWRPSFDY

SEQ ID NO: 50 - protein, 8 aa, Artificial Sequence
  GTC210-04 light chain CDR1
SSNIGNNN

SEQ ID NO: 51 - protein, 3 aa, Artificial Sequence
  GTC210-04 light chain CDR2
SDS

SEQ ID NO: 52 - protein, 11 aa, Artificial Sequence
  GTC210-04 light chain CDR3
GSWDDSLSAYV